European Patent Application EP 4 442 837 A1, published October 9, 2024. Title: 分析方法. Applicant: DENSO CORPORATION. The sequence listing filed with the application follows.

SEQUENCE LISTING (5 sequences)

SEQ ID NO: 1 - DNA, 78 bp, synthetic construct
  source 1..78: mol_type = other DNA
ttttttcagcaccgaccttgtgctttgggagtgctggtccaagggcgttaatggacattttctacatctcagcattct

SEQ ID NO: 2 - DNA, 51 bp, synthetic construct
  source 1..51: mol_type = other DNA
cagcaccgaccttgtgctttgggagtgctggtccaagggcgttaatggaca

SEQ ID NO: 3 - DNA, 18 bp, synthetic construct
  source 1..18: mol_type = other DNA
tctacatctcagcattct

SEQ ID NO: 4 - DNA, 75 bp, synthetic construct
  source 1..75: mol_type = other DNA
gagatgtaccacgaggaaactgtgaagatcgcttcacgagcaacatgaagattgtaggtcacgagtcagaatgct

SEQ ID NO: 5 - DNA, 21 bp, synthetic construct
  source 1..21: mol_type = other DNA
tcacgagcaacatgaagattg